European Patent Application EP 4 410 941 A1, published August 7, 2024. Title: DETERGENT COMPOSITIONS CONTAINING ENZYMES. Applicant: The Procter & Gamble Company. The sequence listing filed with the application follows.

SEQUENCE LISTING (9 sequences)

SEQ ID NO: 1 - protein, 275 aa, Bacillus amyloliquefaciens [sequence omitted]

SEQ ID NO: 2 - DNA, 2188 bp, synthetic construct
  source 1..2188: mol_type = other DNA
gcagttcagcagctgatcatcctgtccacaaaaaagcttgcagaaaaataacattctctgcaagctgatcctgttaaagcttcacaatcactcttccttgaatgcgattttgcaaaatatcttttaacgcacccggcgtttcttccaatgatacttccctgtccacgatggtcagcagctgatcaggcttgagatcagaagacatgcgctcccaaacagcggctctgacgtccatcggacaatatactgaatcgattccgagcaggcttactccgcgaagaataaaaggatacacggttgccggaacttctcctccgccggttaagccgctcactgcgacagatccgccgtattgaattttgcttaaaagcgaggcaagctgttttccgccgactggatcaaccgctccctgccattgctgcttggacagcgccttaagcgttccgtcatagacatcttccctgctgattacttcgcttgcaccaagctgtttcaaataatcagccgcctcccggtttccggtacttgccaccacatcataaccccgcttgttcagcatcgataccgcaattccgccgacaccgccggttgctcctgtgactagcacgctgcctttttccggagacagaccgttctgttcaagccgatgcactgataacgccgcagtaaatcccgccgttccgtacaccatcgcttcttttaacgaaagattctgtggcaaaggcaccagccagtcaccaggcaccgaagcgtattcacttaatccgccatcacgtgagacaccgagctcatagcttgtcgcgatcacctcatccccctccgcaaaacgcggatcattggaagagacgaccgtacccgcagcatcaatgcctaaaataagcggatactctctgacgatattgcctcctgcttttccggccagaccatctttgtaattaatgccggaataagcaactttaatcaggacaccatccttcggcaaatcctctgttgatatggttttcacatggactgaaacatcatcggcatttttttctgcctgcaaggcttgaaataacgttgacattcggcacactccttttcatttatatcgtaaccgaagaacgttcaaaaaaccaaatcatcaagccgccattttcacttcgccggcacattgagacaataatggacaaatccggtatcctcttcatagccgttttgctcatacaagcttcttgccttccggttgtggtgctcagtctgaagtgttaaacattttgccccgttttgccctgcataatcctttgcggcagaaagcagccggccgccggctccctttgtacgcgcatgaggaacgacaaataagtcatttaatatgtatatccttttcattgacacagaagaaaacgttggatagagctgggtaaagcctatgaattctccattttcttctgctatcaaaataacagactcgtgattttccaaacgagctttcaaaaaagcctctgccccttgcaaatcggatgcctgtctataaaattcccgatattggttaaacagcggcgcaatggcggccgcatctgatgtctttgcttggcgaatgttcatcttatttcttcctccctctcaataattttttcattctatcccttttctgtaaagtttatttttcagaatacttttatcatcatgctttgaaaaaatatcacgataatatccattgttctcacggaagcacacgcgctgataaacagctgacatcaactaaaagtttcattaaatactttgaaaaaagttgttgacttaaaagaagctaaatgttatagtaattgtacagaatagtcttttaagtaagtctactctgaatttttttaaaaggagagggtaaagagtgagaagcaaaaaattgtggatcagcttgttgtttgcgttaacgttaatctttacgatggcgttcagcaacatgtctgcgcaggctgcagggaaatcaaacggggaaaagaaatatattgtcgggtttaaacagacaatgagcacgatgagcgccgctaagaagaaagatgtcatttctgaaaaaggcgggaaagtgcaaaagcaattcaaatatgtagacgcagcttcagctacattaaacgaaaaagctgtaaaagaattgaaaaaagacccgagcgtcgcttacgttgaagaagatcacgtagcacatgcgtac

SEQ ID NO: 3 - DNA, 87 bp, Bacillus subtilis
  source 1..87: mol_type = other DNA
gtgagaagcaaaaaattgtggatcagcttgttgtttgcgttaacgttaatctttacgatggcgttcagcaacatgtctgcgcaggct

SEQ ID NO: 4 - DNA, 231 bp, Bacillus amyloliquefaciens
  source 1..231: mol_type = other DNA
gcagggaaatcaaacggggaaaagaaatatattgtcgggtttaaacagacaatgagcacgatgagcgccgctaagaagaaagatgtcatttctgaaaaaggcgggaaagtgcaaaagcaattcaaatatgtagacgcagcttcagctacattaaacgaaaaagctgtaaaagaattgaaaaaagacccgagcgtcgcttacgttgaagaagatcacgtagcacatgcgtac

SEQ ID NO: 5 - DNA, 247 bp, Bacillus amyloliquefaciens
  source 1..247: mol_type = other DNA
acataaaaaaccggccttggccccgccggttttttattatttttcttcctccgcatgttcaatccgctccataatcgacggatggctccctctgaaaattttaacgagaaacggcgggttgacccggctcagtcccgtaacggccaagtcctgaaacgtctcaatcgccgcttcccggtttccggtcagctcaatgccgtaacggtcggcggcgttttcctgataccgggagacggcattcgtaatc

SEQ ID NO: 6 - DNA, 3466 bp, Synthetic construct
  source 1..3466: mol_type = other DNA
tagggcataaggtggtcgcgaatgtgccctgccacgttggacctctagatacataaaaaaccggccttggccccgccggttttttattatttttcttcctccgcatgttcaatccgctccataatcgacggatggctccctctgaaaattttaacgagaaacggcgggttgacccggctcagtcccgtaacggccaagtcctgaaacgtctcaatcgccgcttcccggtttccggtcagctcaatgccgtaacggtcggcggcgttttcctgataccgggagacggcattcgtaatcagtctttcgactgagcctttcgttttatttgatgcctcaagctagagagtcattaccagatctcactgcagtcactactaaaacaattcatccagtaaaatataatattttattttctcccaatcaggcttgatccccagtaagtcaaaaaatagctcgacatactgttcttccccgatatcctccctgatcgaccggacgcagaaggcaatgtcataccacttgtccgccctgccgcttctcccaagatcaataaagccacttactttgccatctttcacaaagatgttgctgtctcccaggtcgccgtgggaaaagacaagttcctcttcgggcttttccgtctttaaaaaatcatacagctcgcgcggatctttaaatggagtgtcttcttcccagttttcgcaatccacatcggccagatcgttattcagtaagtaatccaattcggctaagcggctgtctaagctattcgtatagggacaatccgatatgtcgatggagtgaaagagcctgatgcactccgcatacagctcgataatcttttcagggctttgttcatcttcatactcttccgagcaaaggacgccatcggcctcactcatgagcagattgctccagccatcatgccgttcaaagtgcaggacctttggaacaggcagctttccttccagccatagcatcatgtccttttcccgttccacatcataggtggtccctttataccggctgtccgtcatttttaaatataggttttcattttctcccaccagcttatataccttagcaggagacattccttccgtatcttttacgcagcggtatttttcgatcagttttttcaattccggtgatattctcattttagccatactcatctctccctttttttaaaaatttccccttttaaaattaaaccaaaacccaggagcaaaaacaacacatgatgtatacatcttctttaatccaaaaagaaaatgcttacattaaatcgtttttcaaataaaacaatcgtgcgtttctatataccgttcgatactcgatatgcttaataaagattaagcatatttatattataaacaattatcagacatttgttaaatgtttaactatagttttttttcagccttattctcctgataacgcgagacagcattagaaaaaggcgtaaccgcaaagctcaaaacagaaaacaaaagcaataacagcggaagtgccgcaagatcatgccgcccttctaaatgaaacatgctgcgggttaggcgaaccgtccgcttgtaaagcttatcaatgacataaaatccggcgagcgacacgagcaaatagccagccagaccgatgtaaacgtgcttcatgacataatggcccatttcgtggcccataataaacagaatttctgaatcgtcaagtttgttcagcgtcgtatcccacaatacaatccgtttattggccccaattcctgtaacataggcattcagcgcatttgttttttctgacatgttcacttcatatacatggtcagccggaatattggcttcatctgccagctctaaaattttgctttcaagctctttgtttttcagcggataaaaatcattgtataaaggatcgataatgaccggctgaataaaaaacagaaacagcgaaaacggcactgttaacagccaggcgtataaccaccattttttttcatgccttttgatcagccaataaaaaacgagaacgcaaagcgtaaagattggaaagctgatccaaaagctgataacctgatccttagcccagctggccgttgtctgtgtggaaatgttatagtcaagcgatacttgatagcctatccaatctaaaggcagcgtcaccaatgttgtaatcagcgaaagcacaaacacaaaaccaacggtctgcaaaaaccgaaaaggcacggccgcttcgatccatttcttgattttctttgaaacaccgctgacaagcagaacaaaaaacagaaaccaatcaagtggtaccccgataaaaaataaaaaattcttgacattcgaatactgctcggccactgccaactcagacggcttcatgaaagaagccggatcagcctgcgtccctttcacggcttccggtattgcggaatcacccgacaggaaaaaataccaataaaaaaacagcccgtacagcacgtaagcaagtcctgctgccgcaatccacttgcgcataacgcctcactcctcacatcaacccgttacttctattgtaatcataaattcaaattcttagaaccaagctgtgttccgcacttttccacccttttaagcatggaaaccccgatcgctgggaaaactaacaatgtttggagtgatgcaaatgaaaaaaatagtggcagccatcgtggtaatcggtcttgtgtttatcgcatttttttatctttacagccgatcaggcgatgtgtatcaatcggtagacgcggatttgatcacactgtcttcaagcggccaggaagatatcgagattgaaaaaagacagcacgtcaaagatatgctggatattatgaatcagggaaaacaggtgaagacagaaaaaacatcagcccctgattacgaagggacaatcaagtttcataaagaccggtatgactcattcagactatggattgacggcagccagcaagccgtttttttgaaggatggcacatactacaaattaagcaaaaatgatacaaaggcgctgctaaatattattaaaaaagaagcaaaggattgaaaatgaaaaagcgaagctaaccgcttcgctttttcattttattggggcaaaatatctctcagtgcccgtctgagcattttccccgtcgcatttttcggaatatcgtcaagaaacgtaatggcggcaggccgcttgtattttgccagatgcttttcgcagtgctgcatgatgtcctcctctgttaccccagagcgtttcggcaccacatatccctttaccgcttccccgctttgggggtccggcacgccgatgacaaccgcctccttgacgtccggatggctgtacagcacctcctccacctcccgcggatacacattgtatcctcctacaatgatcatgtcttttttccggtcaacaatgtaaaaatagccgtcctcatcccgtcttgccaagtcccccgtataaagccacccgtctttta

SEQ ID NO: 7 - protein, 275 aa, Synthetic construct
AQSVPYGVSQIKAPALHSQGYTGGNVKVAVIDTGIDSSHPDLKVAGGASMVPGETNPFQDNNSHGTHVAGTVAALDNNIGVLGVAPSASLYAVKVLGADGNGQYSWIINGIEWAIANNMDVINMSLGAPSGSAALKAAVDKAVASGVVVVAAAGNEGTSGSSSTVGYPGKYPSVIAVGAVDSSNQRASFSSVGPELDVMAPGVSIQSTLPGNKYGAQNGTSMASPHVAGAAALILSKHPNWTNTQVRSSLENTTTKLGDSFYYGKGLINVQAAAQ

SEQ ID NO: 8 - protein, 275 aa, Bacillus subtilis
AQSVPYGISQIKAPALHSQGYTGSNVKVAVIDSGIDSSHPDLNVRGGASFVPSETNPYQDGSSHGTHVAGTIAALNNSIGVLGVAPSASLYAVKVLDSTGSGQYSWIINGIEWAISNNMDVINMSLGGPTGSTALKTVVDKAVSSGIVVAAAAGNEGSSGSTSTVGYPAKYPSTIAVGAVNSSNQRASFSSAGSELDVMAPGVSIQSTLPGGTYGAYNGTSMATPHVAGAAALILSKHPTWTNAQVRDRLESTATYLGNSFYYGKGLINVQAAAQ

SEQ ID NO: 9 - protein, 275 aa, Bacillus xiamenensis
AQTVPYGIPQIKAPAVHAQGYKGANVKVAVLDTGIHAAHPDLNVAGGASFVPSEPNATQDFQSHGTHVAGTIAALDNTIGVLGVAPSASLYAVKVLDRNGDGQYSWIISGIEWAVANNMDVINMSLGGPSGSTALKNAVDTANNRGVVVVAAAGNSGSSGSTSTVGYPAKYDSTIAVANVNSNNVRNSSSSAGPELDVSAPGTSILSTVPSSGYASYTGTSMASPHVAGAAALILSKHPNLTNTQVRQRLENTATPLGSSFYYGKGLINVQAAAN